European Patent Specification EP 3 288 964 B1, published February 21, 2024. Title: HIGH THROUGHPUT BH3 PROFILING: A RAPID AND SCALABLE TECHNOLOGY TO BH3 PROFILE ON LOW NUMBERS OF CELLS. Applicant: Dana-Farber Cancer Institute, Inc. Application Not Yet Assigned. The sequence listing filed with the application follows.

SEQUENCE LISTING (17 sequences)

SEQ ID NO: 1 - protein, 20 aa, Artificial Sequence
  Synthetic Polypeptide
  MISC_FEATURE (1)..(1): Modified by Ac
  MOD_RES (20)..(20): AMIDATION
MRPEIWIAQELRRIGDEFNA

SEQ ID NO: 2 - protein, 20 aa, Artificial Sequence
  Synthetic Polypeptide
  MISC_FEATURE (1)..(1): Modified by AC
  MOD_RES (20)..(20): AMIDATION
MRPEIWIAQELRRIGDEFNV

SEQ ID NO: 3 - protein, 20 aa, Artificial Sequence
  Synthetic Polypeptide
EDIIRNIARHLAQVGDSMDR

SEQ ID NO: 4 - protein, 20 aa, Artificial Sequence
  Synthetic Polypeptide
MRPEIWIAQELRRIGDEFNA

SEQ ID NO: 5 - protein, 20 aa, Artificial Sequence [sequence omitted]

SEQ ID NO: 6 - protein, 25 aa, Artificial Sequence
  Synthetic Polypeptide
LWAAQRYGRELRRMSDEFEGSFKGL

SEQ ID NO: 7 - protein, 20 aa, Artificial Sequence
  Synthetic Polypeptide
MEGSDALALRLACIGDEMDV

SEQ ID NO: 8 - protein, 20 aa, Artificial Sequence
  Synthetic Polypeptide
AELPPEFAAQLRKIGDKVYC

SEQ ID NO: 9 - protein, 20 aa, Artificial Sequence
  Synthetic Polypeptide
PADLKDECAQLRRIGDKVNL

SEQ ID NO: 10 - protein, 18 aa, Artificial Sequence
  Synthetic Polypeptide
AAQLTAARLKALGDELHQ

SEQ ID NO: 11 - protein, 20 aa, Artificial Sequence
  Synthetic Polypeptide
EQWAREIGAQLRRMADDLNA

SEQ ID NO: 12 - protein, 20 aa, Artificial Sequence
  Synthetic Polypeptide
HQAEVQIARKLQLIADQFHR

SEQ ID NO: 13 - protein, 25 aa, Artificial Sequence
  Synthetic Polypeptide
NLWAAQRYGRELRRMSDEFVDSFKK

SEQ ID NO: 14 - protein, 25 aa, Artificial Sequence
  Synthetic Polypeptide
LWAAQRYGREARRMSDEFEGSFKGL

SEQ ID NO: 15 - protein, 23 aa, Artificial Sequence
  Synthetic Polypeptide
RPEIWMTQGLRRLGDEINAYYAR

SEQ ID NO: 16 - protein, 20 aa, Artificial Sequence
  Synthetic Polypeptide
EQWAREIGAQARRMAADLNA

SEQ ID NO: 17 - protein, 20 aa, Artificial Sequence
  Synthetic Polypeptide
  misc_feature (1)..(10): Xaa can be any amino acid
  misc_feature (12)..(15): Xaa can be any amino acid
  misc_feature (17)..(20): Xaa can be any amino acid
XXXXXXXXXXLXXXXDXXXX